European Patent Specification EP 3 312 192 B1, published February 22, 2023. Title: Immunogenic compositions containing bacterial outer membrane vesicles and therapeutic uses thereof. Applicant: UNIVERSITA' DEGLI STUDI DI TRENTO. The sequence listing filed with the application follows.

SEQUENCE LISTING (82 sequences)

SEQ ID NO: 1 - DNA, 1680 bp, Artificial Sequence
  recombinant plasmidic DNA
atgaaagctactaaactggtactgggcgcggtaatcctgggttctactctgctggcaggttgcaacaaacaaaacactgctagtacagaaaccacaacgacaaatgagcaaccaaagccagaaagtagtgagctaactactgaaaaagcaggtcagaaaacggatgatatgcttaactctaacgatatgattaagcttgctcccaaagaaatgccactagaatctgcagaaaaagaagaaaaaaagtcagaagacaaaaaaaagagcgaagaagatcacactgaagaaatcaatgacaagatttattcactaaattataatgagcttgaagtacttgctaaaaatggtgaaaccattgaaaattttgttcctaaagaaggcgttaagaaagctgataaatttattgtcattgaaagaaagaaaaaaaatatcaacactacaccagtcgatatttccattattgactctgtcactgataggacctatccagcagcccttcagctggctaataaaggttttaccgaaaacaaaccagacgcggtagtcaccaagcgaaacccacaaaaaatccatattgatttaccaggtatgggagacaaagcaacggttgaggtcaatgaccctacctatgccaatgtttcaacagctattgataatcttgttaaccaatggcatgataattattctggtggtaatacgcttcctgccagaacacaatatactgaatcaatggtatattctaagtcacagattgaggcagctctaaatgttaatagcaaaatcttagatggtactttaggcattgatttcaagtcgatttcaaaaggtgaaaagaaggtgatgattgcagcatacaagcaaattttttacaccgtatcagcaaaccttcctaataatcctgcggatgtgtttgataaatcggtgacctttaaagagttgcaacgaaaaggtgtcagcaatgaagctccgccactctttgtgagtaacgtagcctatggtcgaactgtttttgtcaaactagaaacaagttctaaaagtaatgatgttgaagcggcctttagtgcagctctaaaaggaacagatgttaaaactaatggaaaatattctgatatcttagaaaatagctcatttacagctgtcgttttaggaggagatgctgcagagcacaataaggtagtcacaaaagactttgatgttattagaaacgttatcaaagacaatgctaccttcagtagaaaaaacctagcttatcctatttcatacaccagtgttttccttaaaaataataaaattgcgggtgtcaataacagaactgaatacgttgaaacaacatctaccgagtacactagtggaaaaattaacctgtctcatcaaggcgcgtatgttgctcaatatgaaatcctttgggatgaaatcaattatgatgacaaaggaaaagaagtgattacaaaacgacgttgggacaacaactggtatagtaagacatcaccatttagcacagttatcccactaggagctaattcacgaaatatccgtatcatggctagagagtgcactggcttagctttcgaatggtggcgaaaagtgatcgacgaaagagatgtgaaactgtctaaagaaatcaatgtcaatatctcaggatcaaccttgagcccatatggttcgattacttataagtag

SEQ ID NO: 2 - DNA, 1680 bp, Artificial Sequence
  recombinant plasmidic DNA
atgaaagctactaaactggtactgggcgcggtaatcctgggttctactctgctggcaggtgccaacaaacaaaacactgctagtacagaaaccacaacgacaaatgagcaaccaaagccagaaagtagtgagctaactactgaaaaagcaggtcagaaaacggatgatatgcttaactctaacgatatgattaagcttgctcccaaagaaatgccactagaatctgcagaaaaagaagaaaaaaagtcagaagacaaaaaaaagagcgaagaagatcacactgaagaaatcaatgacaagatttattcactaaattataatgagcttgaagtacttgctaaaaatggtgaaaccattgaaaattttgttcctaaagaaggcgttaagaaagctgataaatttattgtcattgaaagaaagaaaaaaaatatcaacactacaccagtcgatatttccattattgactctgtcactgataggacctatccagcagcccttcagctggctaataaaggttttaccgaaaacaaaccagacgcggtagtcaccaagcgaaacccacaaaaaatccatattgatttaccaggtatgggagacaaagcaacggttgaggtcaatgaccctacctatgccaatgtttcaacagctattgataatcttgttaaccaatggcatgataattattctggtggtaatacgcttcctgccagaacacaatatactgaatcaatggtatattctaagtcacagattgaggcagctctaaatgttaatagcaaaatcttagatggtactttaggcattgatttcaagtcgatttcaaaaggtgaaaagaaggtgatgattgcagcatacaagcaaattttttacaccgtatcagcaaaccttcctaataatcctgcggatgtgtttgataaatcggtgacctttaaagagttgcaacgaaaaggtgtcagcaatgaagctccgccactctttgtgagtaacgtagcctatggtcgaactgtttttgtcaaactagaaacaagttctaaaagtaatgatgttgaagcggcctttagtgcagctctaaaaggaacagatgttaaaactaatggaaaatattctgatatcttagaaaatagctcatttacagctgtcgttttaggaggagatgctgcagagcacaataaggtagtcacaaaagactttgatgttattagaaacgttatcaaagacaatgctaccttcagtagaaaaaacctagcttatcctatttcatacaccagtgttttccttaaaaataataaaattgcgggtgtcaataacagaactgaatacgttgaaacaacatctaccgagtacactagtggaaaaattaacctgtctcatcaaggcgcgtatgttgctcaatatgaaatcctttgggatgaaatcaattatgatgacaaaggaaaagaagtgattacaaaacgacgttgggacaacaactggtatagtaagacatcaccatttagcacagttatcccactaggagctaattcacgaaatatccgtatcatggctagagagtgcactggcttagctttcgaatggtggcgaaaagtgatcgacgaaagagatgtgaaactgtctaaagaaatcaatgtcaatatctcaggatcaaccttgagcccatatggttcgattacttataagtag

SEQ ID NO: 3 - DNA, 882 bp, Artificial Sequence
  recombinant plasmidic DNA
gcagattctgatattaatattaaaaccggtactacagatattggaagcaatactacagtaaaaacaggtgatttagtcacttatgataaagaaaatggcatgttaaaaaaagtattttatagttttatcgatgataaaaatcataataaaaaactgctagttattagaacgaaaggtaccattgctggtcaatatagagtttatagcgaagaaggtgctaacaaaagtggtttagcctggccttcagcctttaaggtacagttgcaactacctgataatgaagtagctcaaatatctgattactatccaagaaattcgattgatacaaaagagtatatgagtactttaacttatggattcaacggtaatgttactggtgatgatacaggaaaaattggcggccttattggtgcaaatgtttcgattggtcatacactgaaatatgttcaacctgatttcaaaacaattttagagagcccaactgataaaaaagtaggctggaaagtgatatttaacaatatggtgaatcaaaattggggaccatatgatagagattcttggaacccggtatatggcaatcaacttttcatgaaaactagaaatggctctatgaaagcagcagataacttccttgatcctaacaaagcaagttctctattatcttcagggttttcaccagacttcgctacagttattactatggatagaaaagcatccaaacaacaaacaaatatagatgtaatatacgaacgagttcgtgatgactaccaattgcactggacttcaacaaattggaaaggtaccaatactaaagataaatggatagatcgttcttcagaaagatataaaatcgattgggaaaaagaagaaatgacaaattaa

SEQ ID NO: 4 - DNA, 945 bp, Artificial Sequence
  recombinant plasmidic DNA
atgaaagctactaaactggtactgggcgcggtaatcctgggttctattttgctggcaggttgcgcagattctgatattaatattaaaaccggtactacagatattggaagcaatactacagtaaaaacaggtgatttagtcacttatgataaagaaaatggcatgctcaaaaaagtattttatagttttatcgatgataaaaatcataataaaaaactgctagttattagaacgaaaggtaccattgctggtcaatatagagtttatagcgaagaaggtgctaacaaaagtggtttagcctggccttcagcctttaaggtacagttgcaactacctgataatgaagtagctcaaatatctgattactatccaagaaattcgattgatacaaaagagtatatgagtactttaacttatggattcaacggtaatgttactggtgatgatacaggaaaaattggcggccttattggtgcaaatgtttcgattggtcatacactgaaatatgttcaacctgatttcaaaacaattttagagagcccaactgataaaaaagtaggctggaaagtgatatttaacaatatggtgaatcaaaattggggaccatatgatagagattcttggaacccggtatatggcaatcaacttttcatgaaaactagaaatggctctatgaaagcagcagataacttccttgatcctaacaaagcaagttctctattatcttcagggttttcaccagacttcgctacagttattactatggatagaaaagcatccaaacaacaaacaaatatagatgtaatatacgaacgagttcgtgatgactaccaattgcactggacttcaacaaattggaaaggtaccaatactaaagataaatggatagatcgttcttcagaaagatataaaatcgattgggaaaaagaagaaatgacaaattaa

SEQ ID NO: 5 - DNA, 947 bp, Artificial Sequence
  recombinant plasmidic DNA
atgatgaaagctactaaactggtactgggcgcggtaatcctgggttctactctgctggcaggtgccgcagattctgatattaatattaaaaccggtactacagatattggaagcaatactacagtaaaaacaggtgatttagtcacttatgataaagaaaatggcatgttaaaaaaagtattttatagttttatcgatgataaaaatcataataaaaaactgctagttattagaacgaaaggtaccattgctggtcaatatagagtttatagcgaagaaggtgctaacaaaagtggtttagcctggccttcagcctttaaggtacagttcaactacctgataatgaagtagctcaaatatctgattactatccaagaaattcgattgatacaaaagagtatatgagtactttaacttatggattcaacggtaatgttactggtgatgatacaggaaaaattggcggccttattggtgcaaatgtttcgattggtcatacactgaaatatgttcaacctgatttcaaaacaattttagagagcccaactgataaaaaagtaggctggaaagtgatatttaacaatatggtgaatcaaaattggggaccatatgatagagattcttggaacccggtatatggcaatcaacttttcatgaaaactagaaatggctctatgaaagcagcagataacttccttgatcctaacaaagcaagttctctattatcttcagggttttcaccagacttcgctacagttattactatggatagaaaagcatccaaacaacaaacaaatatagatgtaatatacgaacgagttcgtgatgactaccaattgcactggacttcaacaaattggaaaggtaccaatactaaagataaatggatagatcgttcttcagaaagatataaaatcgattgggaaaaagaagaaatgacaaattaa

SEQ ID NO: 6 - DNA, 858 bp, Artificial Sequence
  synthetic gene
tgtgggaaccaaggtgaaaaaaataacaaagctgaaactaaatcttataaaatggacgatggcaaaacggtagatattccgaaagaccctaaacgcattgcagtagttgcgccaacatatgctggtggacttaaaaaattaggtgcaaacattgtagctgtaaatcaacaagtcgatcaaagcaaagtattaaaagataaatttaaaggtgttacaaaaattggtgatggcgatgtagaaaaagttgctaaagaaaagccagatttaattattgtatactctactgacaaagatattaaaaaatatcaaaaagtagcaccaacagtagttgttgactataataagcataaatatttagaacaacaagaaatgttagggaaaattgttggtaaagaagataaagtaaaagcttggaagaaagattgggaagaaacaactgctaaagacggtaaagaaattaaaaaagcaattggacaagatgcaacagtgtcattgtttgatgaatttgataaaaaattatacacttacggcgataactggggtcgtggtggagaagtattatatcaagcatttggtttgaaaatgcaaccagaacaacaaaagttaactgcaaaagcaggttgggctgaagtgaaacaagaagaaattgaaaaatatgctggtgattacattgtgagtacaagtgaaggtaaacctacaccaggatacgaatcaacaaacatgtggaagaatttgaaagctactaaagaaggacatattgttaaagttgatgctggtacatactggtacaacgatccttatacattagatttcatgcgtaaagatttaaaagaaaaattaattaaagctgcaaaataa

SEQ ID NO: 7 - DNA, 921 bp, Artificial Sequence
  recombinant plasmidic DNA
atgatgaaagctactaaactggtactgggcgcggtaatcctgggttctactctgctggcaggttgcgggaaccaaggtgaaaaaaataacaaagctgaaactaaatcttataaaatggacgatggcaaaacggtagatattccgaaagaccctaaacgcattgcagtagttgcgccaacatatgctggtggacttaaaaaattaggtgcaaacattgtagctgtaaatcaacaagtcgatcaaagcaaagtattaaaagataaatttaaaggtgttacaaaaattggtgatggcgatgtagaaaaagttgctaaagaaaagccagatttaattattgtatactctactgacaaagatattaaaaaatatcaaaaagtagcaccaacagtagttgttgactataataagcataaatatttagaacaacaagaaatgttagggaaaattgttggtaaagaagataaagtaaaagcttggaagaaagattgggaagaaacaactgctaaagacggtaaagaaattaaaaaagcaattggacaagatgcaacagtgtcattgtttgatgaatttgataaaaaattatacacttacggcgataactggggtcgtggtggagaagtattatatcaagcatttggtttgaaaatgcaaccagaacaacaaaagttaactgcaaaagcaggttgggctgaagtgaaacaagaagaaattgaaaaatatgctggtgattacattgtgagtacaagtgaaggtaaacctacaccaggatacgaatcaacaaacatgtggaagaatttgaaagctactaaagaaggacatattgttaaagttgatgctggtacatactggtacaacgatccttatacattagatttcatgcgtaaagatttaaaagaaaaattaattaaagctgcaaaataa

SEQ ID NO: 8 - DNA, 921 bp, Artificial Sequence
  recombinant plasmidic DNA
atgatgaaagctactaaactggtactgggcgcggtaatcctgggttctactctgctggcaggtgccgggaaccaaggtgaaaaaaataacaaagctgaaactaaatcttataaaatggacgatggcaaaacggtagatattccgaaagaccctaaacgcattgcagtagttgcgccaacatatgctggtggacttaaaaaattaggtgcaaacattgtagctgtaaatcaacaagtcgatcaaagcaaagtattaaaagataaatttaaaggtgttacaaaaattggtgatggcgatgtagaaaaagttgctaaagaaaagccagatttaattattgtatactctactgacaaagatattaaaaaatatcaaaaagtagcaccaacagtagttgttgactataataagcataaatatttagaacaacaagaaatgttagggaaaattgttggtaaagaagataaagtaaaagcttggaagaaagattgggaagaaacaactgctaaagacggtaaagaaattaaaaaagcaattggacaagatgcaacagtgtcattgtttgatgaatttgataaaaaattatacacttacggcgataactggggtcgtggtggagaagtattatatcaagcatttggtttgaaaatgcaaccagaacaacaaaagttaactgcaaaagcaggttgggctgaagtgaaacaagaagaaattgaaaaatatgctggtgattacattgtgagtacaagtgaaggtaaacctacaccaggatacgaatcaacaaacatgtggaagaatttgaaagctactaaagaaggacatattgttaaagttgatgctggtacatactggtacaacgatccttatacattagatttcatgcgtaaagatttaaaagaaaaattaattaaagctgcaaaataa

SEQ ID NO: 9 - DNA, 771 bp, Artificial Sequence
  synthetic gene
atgatgaaacgattaaacaaattagtgttaggcattatttttctgtttttagtcattagtatcactgctggttgtggcataggtaaagaagcggaagttaagaaaagctttgaaaaaacattgagtatgtaccctattaaaaatctagaggatttatacgataaggaaggctatcgtgatgatcagtttgataaaaatgataaaggtacatggattataaattctgaaatggttattcaacctaataatgaagatatggtagctaaaggcatggttctatatatgaatagaaataccaaaacaacaaatggttactactatgtcgatgtgactaaggacgaggatgaaggaaaaccgcacgacaatgaaaaaagatatccggttaaaatggtcgataataaaatcattccaacaaaagaaattaaagatgaaaaaataaaaaaagaaatcgaaaactttaagttctttgttcaatatggcgactttaaaaatttgaaaaattataaagacggagatatttcatataatccagaggtgccgagttattcggctaaatatcaattaactaatgatgattataatgtaaaacaattacgcaaaagatatgatataccgacgagtaaagctccaaagttattgttaaaaggttcagggaatttaaaaggctcatcagttggatataaagatattgaatttacgtttgtagagaaaaaagaagaaaatatatactttagtgatagcttagattataaaaaaagcggagatgtataa

SEQ ID NO: 10 - DNA, 759 bp, Artificial Sequence
  recombinant DNA
atgaaagctactaaactggtactgggcgcggtaatcctgggttctactctgctggcaggttgcggcataggtaaagaagcggaagttaagaaaagctttgaaaaaacattgagtatgtaccctattaaaaatctagaggatttatacgataaggaaggctatcgtgatgatcagtttgataaaaatgataaaggtacatggattataaattctgaaatggttattcaacctaataatgaagatatggtagctaaaggcatggttctatatatgaatagaaataccaaaacaacaaatggttactactatgtcgatgtgactaaggacgaggatgaaggaaaaccgcacgacaatgaaaaaagatatccggttaaaatggtcgataataaaatcattccaacaaaagaaattaaagatgaaaaaataaaaaaagaaatcgaaaactttaagttctttgttcaatatggcgactttaaaaatttgaaaaattataaagacggagatatttcatataatccagaggtgccgagttattcggctaaatatcaattaactaatgatgattataatgtaaaacaattacgcaaaagatatgatataccgacgagtaaagctccaaagttattgttaaaaggttcagggaatttaaaaggctcatcagttggatataaagatattgaatttacgtttgtagagaaaaaagaagaaaatatatactttagtgatagcttagattataaaaaaagcggagatgtataa

SEQ ID NO: 11 - DNA, 759 bp, Artificial Sequence
  recombinant DNA
atgaaagctactaaactggtactgggcgcggtaatcctgggttctactctgctggcaggtgccggcataggtaaagaagcggaagttaagaaaagctttgaaaaaacattgagtatgtaccctattaaaaatctagaggatttatacgataaggaaggctatcgtgatgatcagtttgataaaaatgataaaggtacatggattataaattctgaaatggttattcaacctaataatgaagatatggtagctaaaggcatggttctatatatgaatagaaataccaaaacaacaaatggttactactatgtcgatgtgactaaggacgaggatgaaggaaaaccgcacgacaatgaaaaaagatatccggttaaaatggtcgataataaaatcattccaacaaaagaaattaaagatgaaaaaataaaaaaagaaatcgaaaactttaagttctttgttcaatatggcgactttaaaaatttgaaaaattataaagacggagatatttcatataatccagaggtgccgagttattcggctaaatatcaattaactaatgatgattataatgtaaaacaattacgcaaaagatatgatataccgacgagtaaagctccaaagttattgttaaaaggttcagggaatttaaaaggctcatcagttggatataaagatattgaatttacgtttgtagagaaaaaagaagaaaatatatactttagtgatagcttagattataaaaaaagcggagatgtataa

SEQ ID NO: 12 - DNA, 873 bp, Artificial Sequence
  recombinant DNA
gcacagcatgatgaagccaaaaaaaacgccttttatcaggttctgaatatgccgaatctgaatgccgatcagcgtaatggttttattcagagcctgaaagcagcaccgagccagagcgcaaatgttctgggtgaagcacagaaactgaatgatagccaggcaccgaaagcagatgccaaacgcaacaattttaacaaagataaaaaaagcgcgttttatgaaatcctgaacatgcctaacctgaatgaagcacagcgcaatggctttatccagtctctgaaagccgcaccgtcacagtctaccaatgtgctgggcgaagcgaaaaaactgaacgaatcccaggctccgaaagccgataataacttcaacaaagagaaaaaaaacgccttttatgaaattctgaatatgccaaatctgaacgaagaacagcgtaacggttttattcagtcactgaaagcggctcctagccagtctgcaaatctgctgtctgaagccaaaaaactgaatgaaagtcaggcacctaaagcggataacaaatttaacaaagagaaaaaaaacgcattttatgaaatcctgcatctgccgaatctgaatgaagaacagcgcaacggctttattcagagtctgaaagccgctccgtcccagagcgccaacctgctggccgaagcaaaaaaactgaatgatgcgcaggctccgaaagcagataacaaatttaacaaagagaaaaaaaacgccttctatgaaattctgcacctgcctaacctgaccgaagaacagcgtaatggttttatccagtccctgaaagcggctcctagcgttagcaaagaaatcctggcagaggccaaaaaactgaacgacgcacaggcacctaaa

SEQ ID NO: 13 - DNA, 942 bp, Artificial Sequence
  recombinant DNA
atgatgaaagctactaaactggtactgggcgcggtaatcctgggttctactctgctggcaggttgcgcacagcatgatgaagccaaaaaaaacgccttttatcaggttctgaatatgccgaatctgaatgccgatcagcgtaatggttttattcagagcctgaaagcagcaccgagccagagcgcaaatgttctgggtgaagcacagaaactgaatgatagccaggcaccgaaagcagatgccaaacgcaacaattttaacaaagataaaaaaagcgcgttttatgaaatcctgaacatgcctaacctgaatgaagcacagcgcaatggctttatccagtctctgaaagccgcaccgtcacagtctaccaatgtgctgggcgaagcgaaaaaactgaacgaatcccaggctccgaaagccgataataacttcaacaaagagaaaaaaaacgccttttatgaaattctgaatatgccaaatctgaacgaagaacagcgtaacggttttattcagtcactgaaagcggctcctagccagtctgcaaatctgctgtctgaagccaaaaaactgaatgaaagtcaggcacctaaagcggataacaaatttaacaaagagaaaaaaaacgcattttatgaaatcctgcatctgccgaatctgaatgaagaacagcgcaacggctttattcagagtctgaaagccgctccgtcccagagcgccaacctgctggccgaagcaaaaaaactgaatgatgcgcaggctccgaaagcagataacaaatttaacaaagagaaaaaaaacgccttctatgaaattctgcacctgcctaacctgaccgaagaacagcgtaatggttttatccagtccctgaaagcggctcctagcgttagcaaagaaatcctggcagaggccaaaaaactgaacgacgcacaggcacctaaataa

SEQ ID NO: 14 - DNA, 942 bp, Artificial Sequence
  recombinant DNA
atgatgaaagctactaaactggtactgggcgcggtaatcctgggttctactctgctggcaggtgccgcacagcatgatgaagccaaaaaaaacgccttttatcaggttctgaatatgccgaatctgaatgccgatcagcgtaatggttttattcagagcctgaaagcagcaccgagccagagcgcaaatgttctgggtgaagcacagaaactgaatgatagccaggcaccgaaagcagatgccaaacgcaacaattttaacaaagataaaaaaagcgcgttttatgaaatcctgaacatgcctaacctgaatgaagcacagcgcaatggctttatccagtctctgaaagccgcaccgtcacagtctaccaatgtgctgggcgaagcgaaaaaactgaacgaatcccaggctccgaaagccgataataacttcaacaaagagaaaaaaaacgccttttatgaaattctgaatatgccaaatctgaacgaagaacagcgtaacggttttattcagtcactgaaagcggctcctagccagtctgcaaatctgctgtctgaagccaaaaaactgaatgaaagtcaggcacctaaagcggataacaaatttaacaaagagaaaaaaaacgcattttatgaaatcctgcatctgccgaatctgaatgaagaacagcgcaacggctttattcagagtctgaaagccgctccgtcccagagcgccaacctgctggccgaagcaaaaaaactgaatgatgcgcaggctccgaaagcagataacaaatttaacaaagagaaaaaaaacgccttctatgaaattctgcacctgcctaacctgaccgaagaacagcgtaatggttttatccagtccctgaaagcggctcctagcgttagcaaagaaatcctggcagaggccaaaaaactgaacgacgcacaggcacctaaataa

SEQ ID NO: 15 - DNA, 906 bp, Artificial Sequence
  recombinant DNA
ttgtcagtaggactgattgcacctttagcatctccgattcaagaatctagagcaaatactaatattgaaaatattggtgatggtgctgaagtaatcaaacgtacggaggatgtaagtagtaagaaatggggcgttactcaaaatgtccaattcgactttgtaaaagataaaaaatataacaaagacgctttaattgttaaaatgcaaggttttattaattccagaacttcattttcagatgtgaagggtagtggatatgaattaactaaacgaatgatttggccattccaatataatataggactgacgactaaagatccaaatgttagcttaatcaattaccttcctaaaaacaaaatagaaactactgatgttggtcaaacattaggatataacattggaggtaatttccagtcagcaccatctataggtggcaatggctcatttaattattctaaaacaattagttatacccaaaagagttatgtcagtgaagtagacaagcaaaactcaaaatctgttaaatggggtgttaaagcaaacgaatttgttacgcctgatggaaaaaaatctgcgcatgatagatatttattcgtacaaagtccaaatggtccaacaggttcagcaagagaatattttgctcctgataatcaattgccacctttagttcaaagtggctttaatccatcgtttatcactacactatcacatgaaaaaggttcaagtgatacgagtgaatttgaaatttcatatggtagaaacttagatattacatatgcgactttattccctagaactggtatttacgcagaaagaaagcataatgcatttgtaaatagaaactttgtagttagatatgaagttaattggaaaacacacgaaattaaagtgaaaggacataattaa

SEQ ID NO: 16 - DNA, 918 bp, Artificial Sequence
  recombinant DNA
atgaaagctactaaactggtactgggcgcggtaatcctgggttctactctgctggcaggttgcaatactaatattgaaaatattggtgatggtgctgaagtaatcaaacgtacggaggatgtaagtagtaagaaatggggcgttactcaaaatgtccaattcgactttgtaaaagataaaaaatataacaaagacgctttaattgttaaaatgcaaggttttattaattccagaacttcattttcagatgtgaagggtagtggatatgaattaactaaacgaatgatttggccattccaatataatataggactgacgactaaagatccaaatgttagcttaatcaattaccttcctaaaaacaaaatagaaactactgatgttggtcaaacattaggatataacattggaggtaatttccagtcagcaccatctataggtggcaatggctcatttaattattctaaaacaattagttatacccaaaagagttatgtcagtgaagtagacaagcaaaactcaaaatctgttaaatggggtgttaaagcaaacgaatttgttacgcctgatggaaaaaaatctgcgcatgatagatatttattcgtacaaagtccaaatggtccaacaggttcagcaagagaatattttgctcctgataatcaattgccacctttagttcaaagtggctttaatccatcgtttatcactacactatcacatgaaaaaggttcaagtgatacgagtgaatttgaaatttcatatggtagaaacttagatattacatatgcgactttattccctagaactggtatttacgcagaaagaaagcataatgcatttgtaaatagaaactttgtagttagatatgaagttaattggaaaacacacgaaattaaagtgaaaggacataattaataa

SEQ ID NO: 17 - DNA, 918 bp, Artificial Sequence
  recombinant DNA
atgaaagctactaaactggtactgggcgcggtaatcctgggttctactctgctggcaggtgccaatactaatattgaaaatattggtgatggtgctgaagtaatcaaacgtacggaggatgtaagtagtaagaaatggggcgttactcaaaatgtccaattcgactttgtaaaagataaaaaatataacaaagacgctttaattgttaaaatgcaaggttttattaattccagaacttcattttcagatgtgaagggtagtggatatgaattaactaaacgaatgatttggccattccaatataatataggactgacgactaaagatccaaatgttagcttaatcaattaccttcctaaaaacaaaatagaaactactgatgttggtcaaacattaggatataacattggaggtaatttccagtcagcaccatctataggtggcaatggctcatttaattattctaaaacaattagttatacccaaaagagttatgtcagtgaagtagacaagcaaaactcaaaatctgttaaatggggtgttaaagcaaacgaatttgttacgcctgatggaaaaaaatctgcgcatgatagatatttattcgtacaaagtccaaatggtccaacaggttcagcaagagaatattttgctcctgataatcaattgccacctttagttcaaagtggctttaatccatcgtttatcactacactatcacatgaaaaaggttcaagtgatacgagtgaatttgaaatttcatatggtagaaacttagatattacatatgcgactttattccctagaactggtatttacgcagaaagaaagcataatgcatttgtaaatagaaactttgtagttagatatgaagttaattggaaaacacacgaaattaaagtgaaaggacataattaataa

SEQ ID NO: 18 - DNA, 3128 bp, Artificial Sequence
  recombinant DNA
catcgatttattatgacaacttgacggctacatcattcactttttcttcacaaccggcacggaactcgctcgggctggccccggtgcattttttaaatacccgcgagaaatagagttgatcgtcaaaaccaacattgcgaccgacggtggcgataggcatccgggtggtgctcaaaagcagcttcgcctggctgatacgttggtcctcgcgccagcttaagacgctaatccctaactgctggcggaaaagatgtgacagacgcgacggcgacaagcaaacatgctgtgcgacgctggcgatatcaaaattgctgtctgccaggtgatcgctgatgtactgacaagcctcgcgtacccgattatccatcggtggatggagcgactcgttaatcgcttccatgcgccgcagtaacaattgctcaagcagatttatcgccagcagctccgaatagcgcccttccccttgcccggcgttaatgatttgcccaaacaggtcgctgaaatgcggctggtgcgcttcatccgggcgaaagaaccccgtattggcaaatattgacggccagttaagccattcatgccagtaggcgcgcggacgaaagtaaacccactggtgataccattcgcgagcctccggatgacgaccgtagtgatgaatctctcctggcgggaacagcaaaatatcacccggtcggcaaacaaattctcgtccctgatttttcaccaccccctgaccgcgaatggtgagattgagaatataacctttcattcccagcggtcggtcgataaaaaaatcgagataaccgttggcctcaatcggcgttaaacccgccaccagatgggcattaaacgagtatcccggcagcaggggatcattttgcgcttcagccatacttttcatactcccgccattcagagaagaaaccaattgtccatattgcatcagacattgccgtcactgcgtcttttactggctcttctcgctaaccaaaccggtaaccccgcttattaaaagcattctgtaacaaagcgggaccaaagccatgacaaaaacgcgtaacaaaagtgtctataatcacggcagaaaagtccacattgattatttgcacggcgtcacactttgctatgccatagcatttttatccataagattagcggatcctacctgacgctttttatcgcaactctctactgtttctccatacccgtttttttgggaattcgagctctaaggaggttataaaaaatggatattaatactgaaactgagatcaagcaaaagcattcactaaccccctttcctgttttcctaatcagcccggcatttcgcgggcgatattttcacagctatttcaggagttcagccatgaacgcttattacattcaggatcgtcttgaggctcagagctgggcgcgtcactaccagcagctcgcccgtgaagagaaagaggcagaactggcagacgacatggaaaaaggcctgccccagcacctgtttgaatcgctatgcatcgatcatttgcaacgccacggggccagcaaaaaatccattacccgtgcgtttgatgacgatgttgagtttcaggagcgcatggcagaacacatccggtacatggttgaaaccattgctcaccaccaggttgatattgattcagaggtataaaacgaatgagtactgcactcgcaacgctggctgggaagctggctgaacgtgtcggcatggattctgtcgacccacaggaactgatcaccactcttcgccagacggcatttaaaggtgatgccagcgatgcgcagttcatcgcattactgatcgttgccaaccagtacggccttaatccgtggacgaaagaaatttacgcctttcctgataagcagaatggcatcgttccggtggtgggcgttgatggctggtcccgcatcatcaatgaaaaccagcagtttgatggcatggactttgagcaggacaatgaatcctgtacatgccggatttaccgcaaggaccgtaatcatccgatctgcgttaccgaatggatggatgaatgccgccgcgaaccattcaaaactcgcgaaggcagagaaatcacggggccgtggcagtcgcatcccaaacggatgttacgtcataaagccatgattcagtgtgcccgtctggccttcggatttgctggtatctatgacaaggatgaagccgagcgcattgtcgaaaatactgcatacactgcagaacgtcagccggaacgcgacatcactccggttaacgatgaaaccatgcaggagattaacactctgctgatcgccctggataaaacatgggatgacgacttattgccgctctgttcccagatatttcgccgcgacattcgtgcatcgtcagaactgacacaggccgaagcagtaaaagctcttggattcctgaaacagaaagccgcagagcagaaggtggcagcatgacaccggacattatcctgcagcgtaccgggatcgatgtgagagctgtcgaacagggggatgatgcgtggcacaaattacggctcggcgtcatcaccgcttcagaagttcacaacgtgatagcaaaaccccgctccggaaagaagtggcctgacatgaaaatgtcctacttccacaccctgcttgctgaggtttgcaccggtgtggctccggaagttaacgctaaagcactggcctggggaaaacagtacgagaacgacgccagaaccctgtttgaattcacttccggcgtgaatgttactgaatccccgatcatctatcgcgacgaaagtatgcgtaccgcctgctctcccgatggtttatgcagtgacggcaacggccttgaactgaaatgcccgtttacctcccgggatttcatgaagttccggctcggtggtttcgaggccataaagtcagcttacatggcccaggtgcagtacagcatgtgggtgacgcgaaaaaatgcctggtactttgccaactatgacccgcgtatgaagcgtgaaggcctgcattatgtcgtgattgagcgggatgaaaagtacatggcgagttttgacgagatcgtgccggagttcatcgaaaaaatggacgaggcactggctgaaattggttttgtatttggggagcaatggcgatga

SEQ ID NO: 19 - DNA, 2882 bp, Artificial Sequence
  recombinant DNA
gggcaccaataactgccttaaaaaaaatgattgaacaagatggattgcacgcaggttctccggccgcttgggtggagaggctattcggctatgactgggcacaacagacaatcggctgctctgatgccgccgtgttccggctgtcagcgcaggggcgcccggttctttttgtcaagaccgacctgtccggtgccctgaatgaactgcaggacgaggcagcgcggctatcgtggctggccacgacgggcgttccttgcgcagctgtgctcgacgttgtcactgaagcgggaagggactggctgctattgggcgaagtgccggggcaggatctcctgtcatctcaccttgctcctgccgagaaagtatccatcatggctgatgcaatgcggcggctgcatacgcttgatccggctacctgcccattcgaccaccaagcgaaacatcgcatcgagcgagcacgtactcggatggaagccggtcttgtcgatcaggatgatctggacgaagagcatcaggggctcgcgccagccgaactgttcgccaggctcaaggcgcgcatgcccgacggcgaggatctcgtcgtgacccatggcgatgcctgcttgccgaatatcatggtggaaaatggccgcttttctggattcatcgactgtggccggctgggtgtggcggaccgctatcaggacatagcgttggctacccgtgatattgctgaagagcttggcggcgaatgggctgaccgcttcctcgtgctttacggtatcgccgctcccgattcgcagcgcatcgccttctatcgccttcttgacgagttcttctgatttagcttccttagctcctgaaaatctcgataactcaaaaaatacgcccggtagtgatcttatttcattatggtgaaagttggaacctcttacgtgccgatcaacgtctcacgggatccttaattaagtctagagtcgactgtttaaacctgcagatcctttttaacccatcacatatacctgccgttcactattatttagtgaaatgagatattatgatattttctgaattgtgattaaaaaggcaactttatgcccatgcaacagaaactataaaaaatacagagaatgaaaagaaacagatagattttttagttctttaggcccgtagtctgcaaatccttttatgattttctatcaaacaaaagaggaaaatagaccagttgcaatccaaacgagagtctaatagaatgaggtcgaaaagtaaatcgcgcgggtttgttactgataaagcaggcaagacctaaaatgtgtaaagggcaaagtgtatactttggcgtcaccccttacatattttaggtctttttttattgtgcgtaactaacttgccatcttcaaacaggagggctggaagaagcagaccgctaacacagtacataaaaaaggagacatgaacgatgaacatcaaaaagtttgcaaaacaagcaacagtattaacctttactaccgcactgctggcaggaggcgcaactcaagcgtttgcgaaagaaacgaaccaaaagccatataaggaaacatacggcatttcccatattacacgccatgatatgctgcaaatccctgaacagcaaaaaaatgaaaaatatcaagttcctgaattcgattcgtccacaattaaaaatatctcttctgcaaaaggcctggacgtttgggacagctggccattacaaaacgctgacggcactgtcgcaaactatcacggctaccacatcgtctttgcattagccggagatcctaaaaatgcggatgacacatcgatttacatgttctatcaaaaagtcggcgaaacttctattgacagctggaaaaacgctggccgcgtctttaaagacagcgacaaattcgatgcaaatgattctatcctaaaagaccaaacacaagaatggtcaggttcagccacatttacatctgacggaaaaatccgtttattctacactgatttctccggtaaacattacggcaaacaaacactgacaactgcacaagttaacgtatcagcatcagacagctctttgaacatcaacggtgtagaggattataaatcaatctttgacggtgacggaaaaacgtatcaaaatgtacagcagttcatcgatgaaggcaactacagctcaggcgacaaccatacgctgagagatcctcactacgtagaagataaaggccacaaatacttagtatttgaagcaaacactggaactgaagatggctaccaaggcgaagaatctttatttaacaaagcatactatggcaaaagcacatcattcttccgtcaagaaagtcaaaaacttctgcaaagcgataaaaaacgcacggctgagttagcaaacggcgctctcggtatgattgagctaaacgatgattacacactgaaaaaagtgatgaaaccgctgattgcatctaacacagtaacagatgaaattgaacgcgcgaacgtctttaaaatgaacggcaaatggtacctgttcactgactcccgcggatcaaaaatgacgattgacggcattacgtctaacgatatttacatgcttggttatgtttctaattctttaactggcccatacaagccgctgaacaaaactggccttgtgttaaaaatggatcttgatcctaacgatgtaacctttacttactcacacttcgctgtacctcaagcgaaaggaaacaatgtcgtgattacaagctatatgacaaacagaggattctacgcagacaaacaatcaacgtttgcgccaagcttcctgctgaacatcaaaggcaagaaaacatctgttgtcaaagacagcatccttgaacaaggacaattaacagttaacaaataaaaacgcaaaagaaaatgccgat

SEQ ID NO: 20 - protein, 559 aa, Artificial Sequence
  recombinant protein
MKATKLVLGAVILGSTLLAGCNKQNTASTETTTTNEQPKPESSELTTEKAGQKTDDMLNSNDMIKLAPKEMPLESAEKEEKKSEDKKKSEEDHTEEINDKIYSLNYNELEVLAKNGETIENFVPKEGVKKADKFIVIERKKKNINTTPVDISIIDSVTDRTYPAALQLANKGFTENKPDAVVTKRNPQKIHIDLPGMGDKATVEVNDPTYANVSTAIDNLVNQWHDNYSGGNTLPARTQYTESMVYSKSQIEAALNVNSKILDGTLGIDFKSISKGEKKVMIAAYKQIFYTVSANLPNNPADVFDKSVTFKELQRKGVSNEAPPLFVSNVAYGRTVFVKLETSSKSNDVEAAFSAALKGTDVKTNGKYSDILENSSFTAVVLGGDAAEHNKVVTKDFDVIRNVIKDNATFSRKNLAYPISYTSVFLKNNKIAGVNNRTEYVETTSTEYTSGKINLSHQGAYVAQYEILWDEINYDDKGKEVITKRRWDNNWYSKTSPFSTVIPLGANSRNIRIMARECTGLAFEWWRKVIDERDVKLSKEINVNISGSTLSPYGSITYK

SEQ ID NO: 21 - protein, 559 aa, Artificial Sequence
  recombinant protein
MKATKLVLGAVILGSTLLAGANKQNTASTETTTTNEQPKPESSELTTEKAGQKTDDMLNSNDMIKLAPKEMPLESAEKEEKKSEDKKKSEEDHTEEINDKIYSLNYNELEVLAKNGETIENFVPKEGVKKADKFIVIERKKKNINTTPVDISIIDSVTDRTYPAALQLANKGFTENKPDAVVTKRNPQKIHIDLPGMGDKATVEVNDPTYANVSTAIDNLVNQWHDNYSGGNTLPARTQYTESMVYSKSQIEAALNVNSKILDGTLGIDFKSISKGEKKVMIAAYKQIFYTVSANLPNNPADVFDKSVTFKELQRKGVSNEAPPLFVSNVAYGRTVFVKLETSSKSNDVEAAFSAALKGTDVKTNGKYSDILENSSFTAVVLGGDAAEHNKVVTKDFDVIRNVIKDNATFSRKNLAYPISYTSVFLKNNKIAGVNNRTEYVETTSTEYTSGKINLSHQGAYVAQYEILWDEINYDDKGKEVITKRRWDNNWYSKTSPFSTVIPLGANSRNIRIMARECTGLAFEWWRKVIDERDVKLSKEINVNISGSTLSPYGSITYK

SEQ ID NO: 22 - protein, 293 aa, Artificial Sequence
  recombinant protein
ADSDINIKTGTTDIGSNTTVKTGDLVTYDKENGMLKKVFYSFIDDKNHNKKLLVIRTKGTIAGQYRVYSEEGANKSGLAWPSAFKVQLQLPDNEVAQISDYYPRNSIDTKEYMSTLTYGFNGNVTGDDTGKIGGLIGANVSIGHTLKYVQPDFKTILESPTDKKVGWKVIFNNMVNQNWGPYDRDSWNPVYGNQLFMKTRNGSMKAADNFLDPNKASSLLSSGFSPDFATVITMDRKASKQQTNIDVIYERVRDDYQLHWTSTNWKGTNTKDKWIDRSSERYKIDWEKEEMTN

SEQ ID NO: 23 - protein, 314 aa, Artificial Sequence
  recombinant protein
MKATKLVLGAVILGSILLAGCADSDINIKTGTTDIGSNTTVKTGDLVTYDKENGMLKKVFYSFIDDKNHNKKLLVIRTKGTIAGQYRVYSEEGANKSGLAWPSAFKVQLQLPDNEVAQISDYYPRNSIDTKEYMSTLTYGFNGNVTGDDTGKIGGLIGANVSIGHTLKYVQPDFKTILESPTDKKVGWKVIFNNMVNQNWGPYDRDSWNPVYGNQLFMKTRNGSMKAADNFLDPNKASSLLSSGFSPDFATVITMDRKASKQQTNIDVIYERVRDDYQLHWTSTNWKGTNTKDKWIDRSSERYKIDWEKEEMTN

SEQ ID NO: 24 - protein, 314 aa, Artificial Sequence
  recombinant protein
MKATKLVLGAVILGSTLLAGAADSDINIKTGTTDIGSNTTVKTGDLVTYDKENGMLKKVFYSFIDDKNHNKKLLVIRTKGTIAGQYRVYSEEGANKSGLAWPSAFKVQLQLPDNEVAQISDYYPRNSIDTKEYMSTLTYGFNGNVTGDDTGKIGGLIGANVSIGHTLKYVQPDFKTILESPTDKKVGWKVIFNNMVNQNWGPYDRDSWNPVYGNQLFMKTRNGSMKAADNFLDPNKASSLLSSGFSPDFATVITMDRKASKQQTNIDVIYERVRDDYQLHWTSTNWKGTNTKDKWIDRSSERYKIDWEKEEMTN

SEQ ID NO: 25 - protein, 285 aa, Artificial Sequence
  recombinant protein
CGNQGEKNNKAETKSYKMDDGKTVDIPKDPKRIAVVAPTYAGGLKKLGANIVAVNQQVDQSKVLKDKFKGVTKIGDGDVEKVAKEKPDLIIVYSTDKDIKKYQKVAPTVVVDYNKHKYLEQQEMLGKIVGKEDKVKAWKKDWEETTAKDGKEIKKAIGQDATVSLFDEFDKKLYTYGDNWGRGGEVLYQAFGLKMQPEQQKLTAKAGWAEVKQEEIEKYAGDYIVSTSEGKPTPGYESTNMWKNLKATKEGHIVKVDAGTYWYNDPYTLDFMRKDLKEKLIKAAK

SEQ ID NO: 26 - protein, 305 aa, Artificial Sequence
  recombinant protein
MKATKLVLGAVILGSTLLAGCGNQGEKNNKAETKSYKMDDGKTVDIPKDPKRIAVVAPTYAGGLKKLGANIVAVNQQVDQSKVLKDKFKGVTKIGDGDVEKVAKEKPDLIIVYSTDKDIKKYQKVAPTVVVDYNKHKYLEQQEMLGKIVGKEDKVKAWKKDWEETTAKDGKEIKKAIGQDATVSLFDEFDKKLYTYGDNWGRGGEVLYQAFGLKMQPEQQKLTAKAGWAEVKQEEIEKYAGDYIVSTSEGKPTPGYESTNMWKNLKATKEGHIVKVDAGTYWYNDPYTLDFMRKDLKEKLIKAAK

SEQ ID NO: 27 - protein, 305 aa, Artificial Sequence
  recombinant protein
MKATKLVLGAVILGSTLLAGAGNQGEKNNKAETKSYKMDDGKTVDIPKDPKRIAVVAPTYAGGLKKLGANIVAVNQQVDQSKVLKDKFKGVTKIGDGDVEKVAKEKPDLIIVYSTDKDIKKYQKVAPTVVVDYNKHKYLEQQEMLGKIVGKEDKVKAWKKDWEETTAKDGKEIKKAIGQDATVSLFDEFDKKLYTYGDNWGRGGEVLYQAFGLKMQPEQQKLTAKAGWAEVKQEEIEKYAGDYIVSTSEGKPTPGYESTNMWKNLKATKEGHIVKVDAGTYWYNDPYTLDFMRKDLKEKLIKAAK

SEQ ID NO: 28 - protein, 256 aa, Artificial Sequence
  recombinant protein
MMKRLNKLVLGIIFLFLVISITAGCGIGKEAEVKKSFEKTLSMYPIKNLEDLYDKEGYRDDQFDKNDKGTWIINSEMVIQPNNEDMVAKGMVLYMNRNTKTTNGYYYVDVTKDEDEGKPHDNEKRYPVKMVDNKIIPTKEIKDEKIKKEIENFKFFVQYGDFKNLKNYKDGDISYNPEVPSYSAKYQLTNDDYNVKQLRKRYDIPTSKAPKLLLKGSGNLKGSSVGYKDIEFTFVEKKEENIYFSDSLDYKKSGDV

SEQ ID NO: 29 - protein, 252 aa, Artificial Sequence
  recombinant protein
MKATKLVLGAVILGSTLLAGCGIGKEAEVKKSFEKTLSMYPIKNLEDLYDKEGYRDDQFDKNDKGTWIINSEMVIQPNNEDMVAKGMVLYMNRNTKTTNGYYYVDVTKDEDEGKPHDNEKRYPVKMVDNKIIPTKEIKDEKIKKEIENFKFFVQYGDFKNLKNYKDGDISYNPEVPSYSAKYQLTNDDYNVKQLRKRYDIPTSKAPKLLLKGSGNLKGSSVGYKDIEFTFVEKKEENIYFSDSLDYKKSGDV

SEQ ID NO: 30 - protein, 252 aa, Artificial Sequence
  recombinant protein
MKATKLVLGAVILGSTLLAGAGIGKEAEVKKSFEKTLSMYPIKNLEDLYDKEGYRDDQFDKNDKGTWIINSEMVIQPNNEDMVAKGMVLYMNRNTKTTNGYYYVDVTKDEDEGKPHDNEKRYPVKMVDNKIIPTKEIKDEKIKKEIENFKFFVQYGDFKNLKNYKDGDISYNPEVPSYSAKYQLTNDDYNVKQLRKRYDIPTSKAPKLLLKGSGNLKGSSVGYKDIEFTFVEKKEENIYFSDSLDYKKSGDV

SEQ ID NO: 31 - protein, 291 aa, Artificial Sequence
  recombinant protein
AQHDEAKKNAFYQVLNMPNLNADQRNGFIQSLKAAPSQSANVLGEAQKLNDSQAPKADAKRNNFNKDKKSAFYEILNMPNLNEAQRNGFIQSLKAAPSQSTNVLGEAKKLNESQAPKADNNFNKEKKNAFYEILNMPNLNEEQRNGFIQSLKAAPSQSANLLSEAKKLNESQAPKADNKFNKEKKNAFYEILHLPNLNEEQRNGFIQSLKAAPSQSANLLAEAKKLNDAQAPKADNKFNKEKKNAFYEILHLPNLTEEQRNGFIQSLKAAPSVSKEILAEAKKLNDAQAPK

SEQ ID NO: 32 - protein, 312 aa, Artificial Sequence
  recombinant protein
MKATKLVLGAVILGSTLLAGCAQHDEAKKNAFYQVLNMPNLNADQRNGFIQSLKAAPSQSANVLGEAQKLNDSQAPKADAKRNNFNKDKKSAFYEILNMPNLNEAQRNGFIQSLKAAPSQSTNVLGEAKKLNESQAPKADNNFNKEKKNAFYEILNMPNLNEEQRNGFIQSLKAAPSQSANLLSEAKKLNESQAPKADNKFNKEKKNAFYEILHLPNLNEEQRNGFIQSLKAAPSQSANLLAEAKKLNDAQAPKADNKFNKEKKNAFYEILHLPNLTEEQRNGFIQSLKAAPSVSKEILAEAKKLNDAQAPK

SEQ ID NO: 33 - protein, 312 aa, Artificial Sequence
  recombinant protein
MKATKLVLGAVILGSTLLAGAAQHDEAKKNAFYQVLNMPNLNADQRNGFIQSLKAAPSQSANVLGEAQKLNDSQAPKADAKRNNFNKDKKSAFYEILNMPNLNEAQRNGFIQSLKAAPSQSTNVLGEAKKLNESQAPKADNNFNKEKKNAFYEILNMPNLNEEQRNGFIQSLKAAPSQSANLLSEAKKLNESQAPKADNKFNKEKKNAFYEILHLPNLNEEQRNGFIQSLKAAPSQSANLLAEAKKLNDAQAPKADNKFNKEKKNAFYEILHLPNLTEEQRNGFIQSLKAAPSVSKEILAEAKKLNDAQAPK

SEQ ID NO: 34 - protein, 283 aa, Artificial Sequence
  recombinant protein
NTNIENIGDGAEVIKRTEDVSSKKWGVTQNVQFDFVKDKKYNKDALIVKMQGFINSRTSFSDVKGSGYELTKRMIWPFQYNIGLTTKDPNVSLINYLPKNKIETTDVGQTLGYNIGGNFQSAPSIGGNGSFNYSKTISYTQKSYVSEVDKQNSKSVKWGVKANEFVTPDGKKSAHDRYLFVQSPNGPTGSAREYFAPDNQLPPLVQSGFNPSFITTLSHEKGSSDTSEFEISYGRNLDITYATLFPRTGIYAERKHNAFVNRNFVVRYEVNWKTHEIKVKGHN

SEQ ID NO: 35 - protein, 304 aa, Artificial Sequence
  recombinant protein
MKATKLVLGAVILGSTLLAGCNTNIENIGDGAEVIKRTEDVSSKKWGVTQNVQFDFVKDKKYNKDALIVKMQGFINSRTSFSDVKGSGYELTKRMIWPFQYNIGLTTKDPNVSLINYLPKNKIETTDVGQTLGYNIGGNFQSAPSIGGNGSFNYSKTISYTQKSYVSEVDKQNSKSVKWGVKANEFVTPDGKKSAHDRYLFVQSPNGPTGSAREYFAPDNQLPPLVQSGFNPSFITTLSHEKGSSDTSEFEISYGRNLDITYATLFPRTGIYAERKHNAFVNRNFVVRYEVNWKTHEIKVKGHN

SEQ ID NO: 36 - protein, 304 aa, Artificial Sequence
  recombinant proetin
MKATKLVLGAVILGSTLLAGANTNIENIGDGAEVIKRTEDVSSKKWGVTQNVQFDFVKDKKYNKDALIVKMQGFINSRTSFSDVKGSGYELTKRMIWPFQYNIGLTTKDPNVSLINYLPKNKIETTDVGQTLGYNIGGNFQSAPSIGGNGSFNYSKTISYTQKSYVSEVDKQNSKSVKWGVKANEFVTPDGKKSAHDRYLFVQSPNGPTGSAREYFAPDNQLPPLVQSGFNPSFITTLSHEKGSSDTSEFEISYGRNLDITYATLFPRTGIYAERKHNAFVNRNFVVRYEVNWKTHEIKVKGHN

SEQ ID NO: 37 - DNA, 41 bp, Artificial Sequence
  synthetic oligonucleotide
ggagatatacatatgatgaaagctactaaactggtactggg

SEQ ID NO: 38 - DNA, 35 bp, Artificial Sequence
  synthetic oligonucleotide
gttttgtttgttgctggagcaacctgccagcagag

SEQ ID NO: 39 - DNA, 37 bp, Artificial Sequence
  synthetic oligonucleotide
ggttgctccagcaacaaacaaaacactgctagtacag

SEQ ID NO: 40 - DNA, 41 bp, Artificial Sequence
  synthetic oligonucleotide
gtgatggtgatgttactacttataagtaatcgaaccatatg

SEQ ID NO: 41 - DNA, 30 bp, Artificial Sequence
  synthetic oligonucleotide
catatgtatatctccttcttaaagttaaac

SEQ ID NO: 42 - DNA, 32 bp, Artificial Sequence
  synthetic oligonucleotide
taacatcaccatcaccatcacgattacaaaga

SEQ ID NO: 43 - DNA, 34 bp, Artificial Sequence
  synthetic oligonucleotide
gcaggttgctccagcgcagcagatgagctaagca

SEQ ID NO: 44 - DNA, 39 bp, Artificial Sequence
  synthetic oligonucleotide
gtgatggtgatgttattaggcttttgctgttgctgaggt

SEQ ID NO: 45 - DNA, 23 bp, Artificial Sequence
  synthetic oligonucleotide
gctggagcaacctgccagcagag

SEQ ID NO: 46 - DNA, 45 bp, Artificial Sequence
  synthetic oligonucleotide
ctgctggcaggttgcgcagattctgatattaatattaaaaccggt

SEQ ID NO: 47 - DNA, 45 bp, Artificial Sequence
  synthetic oligonucleotide
gtgatggtgatgttaatttgtcatttcttctttttcccaatcgat

SEQ ID NO: 48 - DNA, 43 bp, Artificial Sequence
  synthetic oligonucleotide
ctgctggcaggttgcgggaaccaaggtgaaaaaaataacaaag

SEQ ID NO: 49 - DNA, 53 bp, Artificial Sequence
  synthetic oligonucleotide
gtgatggtgatgttattttgcagctttaattaatttttcttttaaatctttac

SEQ ID NO: 50 - DNA, 37 bp, Artificial Sequence
  synthetic oligonucleotide
ctgctggcaggttgcggcataggtaaagaagcggaag

SEQ ID NO: 51 - DNA, 44 bp, Artificial Sequence
  synthetic oligonucleotide
gtgatggtgatgttatacatctccgctttttttataatctaagc

SEQ ID NO: 52 - DNA, 39 bp, Artificial Sequence
  synthetic oligonucleotide
ctgctggcaggttgcgcacagcatgatgaagccaaaaaa

SEQ ID NO: 53 - DNA, 36 bp, Artificial Sequence
  synthetic oligonucleotide
gtgatggtgatgttatttaggtgcctgtgcgtcgtt

SEQ ID NO: 54 - DNA, 47 bp, Artificial Sequence
  synthetic oligonucleotide
ctgctggcaggttgcaatactaatattgaaaatattggtgatggtgc

SEQ ID NO: 55 - DNA, 51 bp, Artificial Sequence
  synthetic oligonucleotide
gtgatggtgatgttaattatgtcctttcactttaatttcgtgtgttttcca

SEQ ID NO: 56 - DNA, 30 bp, Artificial Sequence
  synthetic oligonucleotide
caggtgcctccagcaacaaacaaaacactg

SEQ ID NO: 57 - DNA, 27 bp, Artificial Sequence
  synthetic oligonucleotide
caggtgcctccagcgcagcagatgagc

SEQ ID NO: 58 - DNA, 23 bp, Artificial Sequence
  synthetic oligonucleotide
gctggaggcacctgccagcagag

SEQ ID NO: 59 - DNA, 36 bp, Artificial Sequence
  synthetic oligonucleotide
acctgccagcagagtagaacccaggattaccgcgcc

SEQ ID NO: 60 - DNA, 36 bp, Artificial Sequence
  synthetic oligonucleotide
actctgctggcaggtgccggcataggtaaagaagcg

SEQ ID NO: 61 - DNA, 31 bp, Artificial Sequence
  synthetic oligonucleotide
actctgctggcaggtgccgggaaccaaggtg

SEQ ID NO: 62 - DNA, 31 bp, Artificial Sequence
  synthetic oligonucleotide
actctgctggcaggtgccgcacagcatgatg

SEQ ID NO: 63 - DNA, 31 bp, Artificial Sequence
  synthetic oligonucleotide
actctgctggcaggtgccaatactaatattg

SEQ ID NO: 64 - DNA, 33 bp, Artificial Sequence
  synthetic oligonucleotide
actctgctggcaggtgccgcagattctgatatt

SEQ ID NO: 65 - DNA, 35 bp, Artificial Sequence
  synthetic oligonucleotide
aaactgttggctttgaaatgggttacgactggttg

SEQ ID NO: 66 - DNA, 35 bp, Artificial Sequence
  synthetic oligonucleotide
aaaacaaccagtcgtaacccatttcaaagccaaca

SEQ ID NO: 67 - DNA, 35 bp, Artificial Sequence
  synthetic oligonucleotide
aaactcctttcgccacccgcgctactggggagcag

SEQ ID NO: 68 - DNA, 35 bp, Artificial Sequence
  synthetic oligonucleotide
aaaactgctccccagtagcgcgggtggcgaaagga

SEQ ID NO: 69 - DNA, 35 bp, Artificial Sequence
  synthetic oligonucleotide
aaacacaacgtttagagaaaatattgcacaaaccg

SEQ ID NO: 70 - DNA, 35 bp, Artificial Sequence
  synthetic oligonucleotide
aaaacggcatgcacgtttcgcttacgacaaagaaa

SEQ ID NO: 71 - DNA, 120 bp, Artificial Sequence
  synthetic oligonucleotide
accgtgttatctcgttggagatattcatggcgtattttggatgataacgaggcgcaaaaagttctcgtctggtagaaaaaccccgctgctgcggggttttttttgcctttagtaaattga

SEQ ID NO: 72 - DNA, 120 bp, Artificial Sequence
  synthetic oligonucleotide
tcaatttactaaaggcaaaaaaaaccccgcagcagcggggtttttctaccagacgagaactttttgcgcctcgttatcatccaaaatacgccatgaatatctccaacgagataacacggt

SEQ ID NO: 73 - DNA, 120 bp, Artificial Sequence
  synthetic oligonucleotide
caagttgcgccgctacactatcaccagattgatttttgccttatccgaaactggaaaagcaaaagcctctcgcgaggagaggccttcgcctgatgataagttcaagtttgcttcagaata

SEQ ID NO: 74 - DNA, 120 bp, Artificial Sequence
  synthetic oligonucleotide
tattctgaagcaaacttgaacttatcatcaggcgaaggcctctcctcgcgagaggcttttgcttttccagtttcggataaggcaaaaatcaatctggtgatagtgtagcggcgcaacttg

SEQ ID NO: 75 - DNA, 120 bp, Artificial Sequence
  synthetic oligonucleotide
tgttaattgtagctttgctatgctagtagtagatttttgataaatgttttatggtcacaaagttttagtaacttctttaaaatcaatagctaaaataagtaacatcaaaaataacgcgac

SEQ ID NO: 76 - DNA, 120 bp, Artificial Sequence
  synthetic oligonucleotide
gtcgcgttatttttgatgttacttattttagctattgattttaaagaagttactaaaactttgtgaccataaaacatttatcaaaaatctactactagcatagcaaagctacaattaaca

SEQ ID NO: 77 - DNA, 23 bp, Artificial Sequence
  synthetic oligonucleotide
cgttgtagactttacatcgccag

SEQ ID NO: 78 - DNA, 23 bp, Artificial Sequence
  synthetic oligonucleotide
gtcttctctgaagcaggatctgc

SEQ ID NO: 79 - DNA, 22 bp, Artificial Sequence
  synthetic oligonucleotide
gccaaagagattgtgccgcagc

SEQ ID NO: 80 - DNA, 22 bp, Artificial Sequence
  synthetic oligonucleotide
cggtagagtaagtacgttgccg

SEQ ID NO: 81 - DNA, 24 bp, Artificial Sequence
  synthetic oligonucleotide
gcatcatctttaatcgatgcgcgg

SEQ ID NO: 82 - DNA, 23 bp, Artificial Sequence
  synthetic oligonucleotide
gctgtgtcggttaccagtacacc